European Patent Specification EP 3 511 415 B9, published August 20, 2025. Title: TRYPTOPHAN OXIDASE AND USE THEREOF. Applicant: AJINOMOTO CO., INC. The sequence listing filed with the application follows.

SEQUENCE LISTING (4 sequences)

SEQ ID NO: 1 - DNA, 1254 bp, Chromobacterium violaceum
atgaagcattcttccgatatctgcattgtcggcgccggcatcagcggcctgacctgcgccagccatctgctcgactcgcccgcttgccgcggcctgtcgctgcgcatcttcgacatgcagcaggaggcgggcggccgcatccgctcgaagatgctggatggcaaggcgtcgatagagctgggcgcggggcgatactccccgcagctgcacccgcatttccagagcgcgatgcagcattacagccagaagagcgaggtgtatccgttcacccagctgaaattcaagagccatgtccagcagaagctgaagcgggcgatgaacgagttgtcgcccaggctgaaagagcatggcaaggaatcctttctccagttcgtcagccgctaccagggccatgacagcgcggtgggcatgatccgctccatgggctacgacgcgctgttcctgcccgacatctcggccgagatggcctacgacatcgtcggcaagcacccggaaatccagagcgtgaccgataacgacgccaaccagtggttcgcggcggaaacgggctttgcgggcctgatccagggcatcaaggccaaggtcaaggctgccggcgcgcgcttcagcctgggttaccggctgctgtcggtgaggacggacggcgacggctacctgctgcaactggccggcgacgacggctggaagctggaacaccggacccgccatctgatcctggccattcctccgtcggcgatggccgggctcaatgtcgacttccccgaggcgtggagcggcgcgcgctacggctcgctgccgctgttcaagggtttcctcacctacggcgagccatggtggctggactacaagctggacgaccaggtgctgatcgtcgacaacccgctgcgcaagatctacttcaagggcgacaagtacctgttcttctacaccgacagcgagatggccaattactggcgcggctgcgtggccgaaggagaggacggctacctggagcagatccgcacccatctggccagcgcgctgggcatcgttcgcgagcgcattccccagcccctcgcccatgtgcacaagtattgggcgcatggcgtggagttctgccgcgacagcgatatcgaccatccgtccgcgctcagccaccgcgacagcggcatcatcgcctgttcggacgcctacaccgagcactgcggctggatggagggcggcctgctcagcgcccgcgaagccagccgtctgctgctgcagcgcatcgccgcg

SEQ ID NO: 2 - protein, 418 aa, Chromobacterium violaceum
MKHSSDICIVGAGISGLTCASHLLDSPACRGLSLRIFDMQQEAGGRIRSKMLDGKASIELGAGRYSPQLHPHFQSAMQHYSQKSEVYPFTQLKFKSHVQQKLKRAMNELSPRLKEHGKESFLQFVSRYQGHDSAVGMIRSMGYDALFLPDISAEMAYDIVGKHPEIQSVTDNDANQWFAAETGFAGLIQGIKAKVKAAGARFSLGYRLLSVRTDGDGYLLQLAGDDGWKLEHRTRHLILAIPPSAMAGLNVDFPEAWSGARYGSLPLFKGFLTYGEPWWLDYKLDDQVLIVDNPLRKIYFKGDKYLFFYTDSEMANYWRGCVAEGEDGYLEQIRTHLASALGIARERIPQPLAHVHKYWAHGVEFCRDSDIDHPSALSHRDSGIIACSDAYTEHCGWMEGGLLSAREASRLLLQRIAA

SEQ ID NO: 3 - DNA, 53 bp, Artificial Sequence
  Primer for amplifying TrpOX gene
gagatatacatatgcatcaccatcaccatcacaagcattcttccgatatctgc

SEQ ID NO: 4 - DNA, 37 bp, Artificial Sequence
  Primer for amplifying TrpOX gene
gctgctgcagcgcatcgccgcgtaatgaaagcttgcg